European Patent Specification EP 3 789 491 B1, published April 16, 2025. Title: PEPTIDE AND USE THEREOF. Applicant: NIIGATA UNIVERSITY. The sequence listing filed with the application follows.

SEQUENCE LISTING (47 sequences)

SEQ ID NO: 1 - protein, 9 aa, Artificial Sequence
  Synthesized
  MISC_FEATURE (2)..(2): Xaa indicates Arg or Methyl-Arg.
RXPTTWHKP

SEQ ID NO: 2 - protein, 9 aa, Artificial Sequence
  Synthesized
  MISC_FEATURE (2)..(2): Xaa indicates Arg or Methyl-Arg.
  MISC_FEATURE (3)..(3): Xaa indicates Arg or Methyl-Arg.
AXXYTWIRA

SEQ ID NO: 3 - protein, 9 aa, Artificial Sequence
  Synthesized
  MISC_FEATURE (2)..(2): Xaa indicates Ala or Methyl-Ala.
RXWRQCRWR

SEQ ID NO: 4 - protein, 9 aa, Artificial Sequence
  Synthesized
RRPTTWHKP

SEQ ID NO: 5 - protein, 9 aa, Artificial Sequence
  Synthesized
  MISC_FEATURE (2)..(2): Xaa indicates Methyl-Arg.
RXPTTWHKP

SEQ ID NO: 6 - protein, 9 aa, Artificial Sequence
  Synthesized
ARRYTWIRA

SEQ ID NO: 7 - protein, 9 aa, Artificial Sequence
  Synthesized
  MISC_FEATURE (2)..(2): Xaa indicates Methyl-Arg.
AXRYTWIRA

SEQ ID NO: 8 - protein, 9 aa, Artificial Sequence
  Synthesized
  MISC_FEATURE (3)..(3): Xaa indicates Methyl-Arg.
ARXYTWIRA

SEQ ID NO: 9 - protein, 9 aa, Artificial Sequence
  Synthesized
  MISC_FEATURE (2)..(2): Xaa indicates Methyl-Arg.
  MISC_FEATURE (3)..(3): Xaa indicates Methyl-Arg.
AXXYTWIRA

SEQ ID NO: 10 - protein, 9 aa, Artificial Sequence
  Synthesized
RAWRQCRWR

SEQ ID NO: 11 - protein, 9 aa, Artificial Sequence
  Synthesized
  MISC_FEATURE (2)..(2): Xaa indicates Methyl-Ala.
RXWRQCRWR

SEQ ID NO: 12 - protein, 6 aa, Artificial Sequence
  Synthesized
RPTTWH

SEQ ID NO: 13 - protein, 8 aa, Artificial Sequence
  Synthesized
RPTTWHKP

SEQ ID NO: 14 - protein, 7 aa, Artificial Sequence
  Synthesized
RRPTTWH

SEQ ID NO: 15 - protein, 19 aa, Artificial Sequence
  Synthesized
RRPTTWHKPGRRPTTWHKP

SEQ ID NO: 16 - protein, 29 aa, Artificial Sequence
  Synthesized
RRPTTWHKPGRRPTTWHKPGRRPTTWHKP

SEQ ID NO: 17 - protein, 19 aa, Artificial Sequence
  Synthesized
RRPTTWHKPGPKHWTTPRR

SEQ ID NO: 18 - protein, 19 aa, Artificial Sequence
  Synthesized
  MISC_FEATURE (2)..(2): Xaa indicates Methyl-Arg.
RXPTTWHKPGRRPTTWHKP

SEQ ID NO: 19 - protein, 19 aa, Artificial Sequence
  Synthesized
  MISC_FEATURE (2)..(2): Xaa indicates Methyl-Arg.
RXPTTWHKPGPKHWTTPRR

SEQ ID NO: 20 - protein, 17 aa, Artificial Sequence
  Synthesized
RPTTWHKPGRPTTWHKP

SEQ ID NO: 21 - protein, 18 aa, Artificial Sequence
  Synthesized
RPTTWHKPGRRPTTWHKP

SEQ ID NO: 22 - protein, 15 aa, Artificial Sequence
  Synthesized
RRPTTWHGRRPTTWH

SEQ ID NO: 23 - protein, 17 aa, Artificial Sequence
  Synthesized
RRPTTWHGRRPTTWHKP

SEQ ID NO: 24 - protein, 17 aa, Artificial Sequence
  Synthesized
RRPTTWHKPGRRPTTWH

SEQ ID NO: 25 - protein, 17 aa, Artificial Sequence
  Synthesized
  MISC_FEATURE (2)..(2): Xaa indicates Methyl-Arg.
RXPTTWHKPGRRPTTWH

SEQ ID NO: 26 - protein, 17 aa, Artificial Sequence
  Synthesized
  MISC_FEATURE (2)..(2): Xaa indicates Methyl-Arg.
RXPTTWHGRRPTTWHKP

SEQ ID NO: 27 - protein, 19 aa, Artificial Sequence
  Synthesized
  MISC_FEATURE (2)..(2): Xaa indicates Methyl-Arg.
RXPTTWHKPCRRPTTWHKP

SEQ ID NO: 28 - protein, 29 aa, Artificial Sequence
  Synthesized
  MISC_FEATURE (2)..(2): Xaa indicates Methyl-Arg.
RXPTTWHKPCRRPTTWHKPGRRPTTWHKP

SEQ ID NO: 29 - protein, 28 aa, Artificial Sequence
  Synthesized
RPTTWHKPGRRPTTWHKPCRRPTTWHKP

SEQ ID NO: 30 - protein, 28 aa, Artificial Sequence
  Synthesized
RPTTWHKPCRRPTTWHKPCRRPTTWHKP

SEQ ID NO: 31 - protein, 28 aa, Artificial Sequence
  Synthesized
RPTTWHKPGRRPTTWHKPKRRPTTWHKP

SEQ ID NO: 32 - DNA, 57 bp, Artificial Sequence
  Synthesized
cggcggccgactacgtggcataagcctgggcggcggccgactacgtggcataagcct

SEQ ID NO: 33 - DNA, 87 bp, Artificial Sequence
  Synthesized
cggcggccgactacgtggcataagcctgggcggcggccgactacgtggcataagcctgggcggcggccgactacgtggcataagcct

SEQ ID NO: 34 - DNA, 57 bp, Artificial Sequence
  Synthesized
cggcggccgactacgtggcataagcctgggcctaagcattggacgactccgcggcgg

SEQ ID NO: 35 - protein, 6 aa, Artificial Sequence
  Synthesized
TTWHKP

SEQ ID NO: 36 - protein, 4 aa, Artificial Sequence
  Synthesized
TTWH

SEQ ID NO: 37 - protein, 3 aa, Artificial Sequence
  Synthesized
TWH

SEQ ID NO: 38 - protein, 2 aa, Artificial Sequence
  Synthesized
WH

SEQ ID NO: 39 - protein, 16 aa, Artificial Sequence
  Synthesized
TTWHKPGRRPTTWHKP

SEQ ID NO: 40 - protein, 18 aa, Artificial Sequence
  Synthesized
RPTTWHKPGPKHWTTPRR

SEQ ID NO: 41 - protein, 16 aa, Artificial Sequence
  Synthesized
TTWHKPGPKHWTTPRR

SEQ ID NO: 42 - protein, 23 aa, Artificial Sequence
  Synthesized
CGGGRRPTTWHKPGRRPTTWHKP

SEQ ID NO: 43 - protein, 5 aa, Artificial Sequence
  Synthesized
RPTTW

SEQ ID NO: 44 - protein, 5 aa, Artificial Sequence
  Synthesized
PTTWH

SEQ ID NO: 45 - protein, 9 aa, Artificial Sequence
  Synthesized
PKHWTTPRR

SEQ ID NO: 46 - protein, 21 aa, Artificial Sequence
  Synthesized
RRPTTWHKPGPGRRPTTWHKP

SEQ ID NO: 47 - protein, 19 aa, Artificial Sequence
  Synthesized
PKHWTTPRRGPKHWTTPRR